European Patent Specification EP 3 645 551 B1, published March 13, 2024. Title: Tropism-Modified Recombinant Viral Vectors and Uses Thereof for the Targeted Introduction of Genetic Material into Human Cell. Applicant: Regeneron Pharmaceuticals, Inc. Kyratsous, Christos Murphy, Andrew J Wang, Cheng Sabin, Leah. The sequence listing filed with the application follows.

SEQUENCE LISTING (40 sequences)

SEQ ID NO: 1 - protein, 735 aa, adeno-associated virus 2 [sequence omitted]

SEQ ID NO: 2 - protein, 745 aa, Artificial Sequence
  AAV2 VP1 N587Myc
MAADGYLPDWLEDTLSEGIRQWWKLKPGPPPPKPAERHKDDSRGLVLPGYKYLGPFNGLDKGEPVNEADAAALEHDKAYDRQLDSGDNPYLKYNHADAEFQERLKEDTSFGGNLGRAVFQAKKRVLEPLGLVEEPVKTAPGKKRPVEHSPVEPDSSSGTGKAGQQPARKRLNFGQTGDADSVPDPQPLGQPPAAPSGLGTNTMATGSGAPMADNNEGADGVGNSSGNWHCDSTWMGDRVITTSTRTWALPTYNNHLYKQISSQSGASNDNHYFGYSTPWGYFDFNRFHCHFSPRDWQRLINNNWGFRPKRLNFKLFNIQVKEVTQNDGTTTIANNLTSTVQVFTDSEYQLPYVLGSAHQGCLPPFPADVFMVPQYGYLTLNNGSQAVGRSSFYCLEYFPSQMLRTGNNFTFSYTFEDVPFHSSYAHSQSLDRLMNPLIDQYLYYLSRTNTPSGTTTQSRLQFSQAGASDIRDQSRNWLPGPCYRQQRVSKTSADNNNSEYSWTGATKYHLNGRDSLVNPGPAMASHKDDEEKFFPQSGVLIFGKQGSEKTNVDIEKVMITDEEEIRTTNPVATEQYGSVSTNLQRGNEQKLISEEDLRQAATADVNTQGVLPGMVWQDRDVYLQGPIWAKIPHTDGHFHPSPLMGGFGLKHPPPQILIKNTPVPANPSTTFSAAKFASFITQYSTGQVSVEIEWELQKENSKRWNPEIQYTSNYNKSVNVDFTVDTNGVYSEPRPIGTRYLTRNL

SEQ ID NO: 3 - protein, 736 aa, adeno-associated virus 6
MAADGYLPDWLEDNLSEGIREWWDLKPGAPKPKANQQKQDDGRGLVLPGYKYLGPFNGLDKGEPVNAADAAALEHDKAYDQQLKAGDNPYLRYNHADAEFQERLQEDTSFGGNLGRAVFQAKKRVLEPFGLVEEGAKTAPGKKRPVEQSPQEPDSSSGIGKTGQQPAKKRLNFGQTGDSESVPDPQPLGEPPATPAAVGPTTMASGGGAPMADNNEGADGVGNASGNWHCDSTWLGDRVITTSTRTWALPTYNNHLYKQISSASTGASNDNHYFGYSTPWGYFDFNRFHCHFSPRDWQRLINNNWGFRPKRLNFKLFNIQVKEVTTNDGVTTIANNLTSTVQVFSDSEYQLPYVLGSAHQGCLPPFPADVFMIPQYGYLTLNNGSQAVGRSSFYCLEYFPSQMLRTGNNFTFSYTFEDVPFHSSYAHSQSLDRLMNPLIDQYLYYLNRTQNQSGSAQNKDLLFSRGSPAGMSVQPKNWLPGPCYRQQRVSKTKTDNNNSNFTWTGASKYNLNGRESIINPGTAMASHKDDKDKFFPMSGVMIFGKESAGASNTALDNVMITDEEEIKATNPVATERFGTVAVNLQSSSTDPATGDVHVMGALPGMVWQDRDVYLQGPIWAKIPHTDGHFHPSPLMGGFGLKHPPPQILIKNTPVPANPPAEFSATKFASFITQYSTGQVSVEIEWELQKENSKRWNPEVQYTSNYAKSANVDFTVDNNGLYTEPRPIGTRYLTRPL

SEQ ID NO: 4 - protein, 746 aa, Artificial Sequence
  AAV6 VP1 Q585Myc
MAADGYLPDWLEDNLSEGIREWWDLKPGAPKPKANQQKQDDGRGLVLPGYKYLGPFNGLDKGEPVNAADAAALEHDKAYDQQLKAGDNPYLRYNHADAEFQERLQEDTSFGGNLGRAVFQAKKRVLEPFGLVEEGAKTAPGKKRPVEQSPQEPDSSSGIGKTGQQPAKKRLNFGQTGDSESVPDPQPLGEPPATPAAVGPTTMASGGGAPMADNNEGADGVGNASGNWHCDSTWLGDRVITTSTRTWALPTYNNHLYKQISSASTGASNDNHYFGYSTPWGYFDFNRFHCHFSPRDWQRLINNNWGFRPKRLNFKLFNIQVKEVTTNDGVTTIANNLTSTVQVFSDSEYQLPYVLGSAHQGCLPPFPADVFMIPQYGYLTLNNGSQAVGRSSFYCLEYFPSQMLRTGNNFTFSYTFEDVPFHSSYAHSQSLDRLMNPLIDQYLYYLNRTQNQSGSAQNKDLLFSRGSPAGMSVQPKNWLPGPCYRQQRVSKTKTDNNNSNFTWTGASKYNLNGRESIINPGTAMASHKDDKDKFFPMSGVMIFGKESAGASNTALDNVMITDEEEIKATNPVATERFGTVAVNLQEQKLISEEDLSSSTDPATGDVHVMGALPGMVWQDRDVYLQGPIWAKIPHTDGHFHPSPLMGGFGLKHPPPQILIKNTPVPANPPAEFSATKFASFITQYSTGQVSVEIEWELQKENSKRWNPEVQYTSNYAKSANVDFTVDNNGLYTEPRPIGTRYLTRPL

SEQ ID NO: 5 - protein, 736 aa, adeno-associated virus 9
MAADGYLPDWLEDNLSEGIREWWALKPGAPQPKANQQHQDNARGLVLPGYKYLGPGNGLDKGEPVNAADAAALEHDKAYDQQLKAGDNPYLKYNHADAEFQERLKEDTSFGGNLGRAVFQAKKRLLEPLGLVEEAAKTAPGKKRPVEQSPQEPDSSAGIGKSGAQPAKKRLNFGQTGDTESVPDPQPIGEPPAAPSGVGSLTMASGGGAPVADNNEGADGVGSSSGNWHCDSQWLGDRVITTSTRTWALPTYNNHLYKQISNSTSGGSSNDNAYFGYSTPWGYFDFNRFHCHFSPRDWQRLINNNWGFRPKRLNFKLFNIQVKEVTDNNGVKTIANNLTSTVQVFTDSDYQLPYVLGSAHEGCLPPFPADVFMIPQYGYLTLNDGSQAVGRSSFYCLEYFPSQMLRTGNNFQFSYEFENVPFHSSYAHSQSLDRLMNPLIDQYLYYLSKTINGSGQNQQTLKFSVAGPSNMAVQGRNYIPGPSYRQQRVSTTVTQNNNSEFAWPGASSWALNGRNSLMNPGPAMASHKEGEDRFFPLSGSLIFGKQGTGRDNVDADKVMITNEEEIKTTNPVATESYGQVATNHQSAQAQAQTGWVQNQGILPGMVWQDRDVYLQGPIWAKIPHTDGNFHPSPLMGGFGMKHPPPQILIKNTPVPADPPTAFNKDKLNSFITQYSTGQVSVEIEWELQKENSKRWNPEIQYTSNYYKSNNVEFAVNTEGVYSEPRPIGTRYLTRNL

SEQ ID NO: 6 - protein, 10 aa, Artificial Sequence
  c-myc
EQKLISEEDL

SEQ ID NO: 7 - protein, 8 aa, Artificial Sequence
  FLAG
DYKDDDDK

SEQ ID NO: 8 - protein, 9 aa, Artificial Sequence
  HA
YPYDVPDYA

SEQ ID NO: 9 - DNA, 21 bp, Artificial Sequence
  Fwd ITR primer
ggaacccctagtgatggagtt

SEQ ID NO: 10 - DNA, 16 bp, Artificial Sequence
  Rvs ITR primer
cggcctcagtgagcga

SEQ ID NO: 11 - DNA, 21 bp, Artificial Sequence
  AAV2 ITRs probe
cactccctctctgcgcgctcg

SEQ ID NO: 12 - DNA, 30 bp, Artificial Sequence
  c-myc
gaacaaaaactcatctcagaagaggatctg

SEQ ID NO: 13 - DNA, 20 bp, Artificial Sequence
  pAAVRCBsiWF
ggagtaccagctcccgtacg

SEQ ID NO: 14 - DNA, 43 bp, Artificial Sequence
  N587mycR
ctcttctgagatgagtttttgttcgttgcctctctggaggttg

SEQ ID NO: 15 - DNA, 43 bp, Artificial Sequence
  N587mycF
aaactcatctcagaagaggatctgagacaagcagctaccgcag

SEQ ID NO: 16 - DNA, 18 bp, Artificial Sequence
  pAAVRCPmeR
tccgcccgctgtttaaac

SEQ ID NO: 17 - DNA, 24 bp, Artificial Sequence
  pAAVRC9BsiWF
actcagactatcagctcccgtacg

SEQ ID NO: 18 - DNA, 41 bp, Artificial Sequence
  A589mycR
ctcttctgagatgagtttttgttctgcttgggcactctggt

SEQ ID NO: 19 - DNA, 37 bp, Artificial Sequence
  A589mycF
aaactcatctcagagaggatctgcaggcgcagaccgg

SEQ ID NO: 20 - DNA, 19 bp, Artificial Sequence
  pAAVRC9PmeR
ctccgcccgctgtttaaac

SEQ ID NO: 21 - protein, 738 aa, adeno-associated virus 8
MAADGYLPDWLEDNLSEGIREWWALKPGAPKPKANQQKQDDGRGLVLPGYKYLGPFNGLDKGEPVNAADAAALEHDKAYDQQLQAGDNPYLRYNHADAEFQERLQEDTSFGGNLGRAVFQAKKRVLEPLGLVEEGAKTAPGKKRPVEPSPQRSPDSSTGIGKKGQQPARKRLNFGQTGDSESVPDPQPLGEPPAAPSGVGPNTMAAGGGAPMADNNEGADGVGSSSGNWHCDSTWLGDRVITTSTRTWALPTYNNHLYKQISNGTSGGATNDNTYFGYSTPWGYFDFNRFHCHFSPRDWQRLINNNWGFRPKRLSFKLFNIQVKEVTQNEGTKTIANNLTSTIQVFTDSEYQLPYVLGSAHQGCLPPFPADVFMIPQYGYLTLNNGSQAVGRSSFYCLEYFPSQMLRTGNNFQFTYTFEDVPFHSSYAHSQSLDRLMNPLIDQYLYYLSRTQTTGGTANTQTLGFSQGGPNTMANQAKNWLPGPCYRQQRVSTTTGQNNNSNFAWTAGTKYHLNGRNSLANPGIAMATHKDDEERFFPSNGILIFGKQNAARDNADYSDVMLTSEEEIKTTNPVATEEYGIVADNLQQQNTAPQIGTVNSQGALPGMVWQNRDVYLQGPIWAKIPHTDGNFHPSPLMGGFGLKHPPPQILIKNTPVPADPPTTFNQSKLNSFITQYSTGQVSVEIEWELQKENSKRWNPEIQYTSNYYKSTSVDFAVNTEGVYSEPRPIGTRYLTRNL

SEQ ID NO: 22 - DNA, 453 bp, Artificial Sequence
  AAV8 N590myc gblock
gaccctgttaccgccaacaacgcgtctcaacgacaaccgggcaaaacaacaatagcaactttgcctggactgctgggaccaaataccatctgaatggaagaaattcattggctaatcctggcatcgctatggcaacacacaaagacgacgaggagcgtttttttcccagtaacgggatcctgatttttggcaaacaaaatgctgccagagacaatgcggattacagcgatgtcatgctcaccagcgaggaagaaatcaaaaccactaaccctgtggctacagaggaatacggtatcgtggcagataacttgcagcagcaaaacgaacaaaaactcatctcagaagaggatctgacggctcctcaaattggaactgtcaacagccagggggccttacccggtatggtctggcagaaccgggacgtgtacctgcagggtcccatctgggccaaga

SEQ ID NO: 23 - DNA, 7336 bp, Artificial Sequence
  pAAV RC2/8
gcgcgccgatatcgttaacgccccgcgccggccgctctagaactagtggatcccccggaagatcagaagttcctattccgaagttcctattctctagaaagtataggaacttctgatctgcgcagccgccatgccggggttttacgagattgtgattaaggtccccagcgaccttgacgagcatctgcccggcatttctgacagctttgtgaactgggtggccgagaaggaatgggagttgccgccagattctgacatggatctgaatctgattgagcaggcacccctgaccgtggccgagaagctgcagcgcgactttctgacggaatggcgccgtgtgagtaaggccccggaggcccttttctttgtgcaatttgagaagggagagagctacttccacatgcacgtgctcgtggaaaccaccggggtgaaatccatggttttgggacgtttcctgagtcagattcgcgaaaaactgattcagagaatttaccgcgggatcgagccgactttgccaaactggttcgcggtcacaaagaccagaaatggcgccggaggcgggaacaaggtggtggatgagtgctacatccccaattacttgctccccaaaacccagcctgagctccagtgggcgtggactaatatggaacagtatttaagcgcctgtttgaatctcacggagcgtaaacggttggtggcgcagcatctgacgcacgtgtcgcagacgcaggagcagaacaaagagaatcagaatcccaattctgatgcgccggtgatcagatcaaaaacttcagccaggtacatggagctggtcgggtggctcgtggacaaggggattacctcggagaagcagtggatccaggaggaccaggcctcatacatctccttcaatgcggcctccaactcgcggtcccaaatcaaggctgccttggacaatgcgggaaagattatgagcctgactaaaaccgcccccgactacctggtgggccagcagcccgtggaggacatttccagcaatcggatttataaaattttggaactaaacgggtacgatccccaatatgcggcttccgtctttctgggatgggccacgaaaaagttcggcaagaggaacaccatctggctgtttgggcctgcaactaccgggaagaccaacatcgcggaggccatagcccacactgtgcccttctacgggtgcgtaaactggaccaatgagaactttcccttcaacgactgtgtcgacaagatggtgatctggtgggaggaggggaagatgaccgccaaggtcgtggagtcggccaaagccattctcggaggaagcaaggtgcgcgtggaccagaaatgcaagtcctcggcccagatagacccgactcccgtgatcgtcacctccaacaccaacatgtgcgccgtgattgacgggaactcaacgaccttcgaacaccagcagccgttgcaagaccggatgttcaaatttgaactcacccgccgtctggatcatgactttgggaaggtcaccaagcaggaagtcaaagactttttccggtgggcaaaggatcacgtggttgaggtggagcatgaattctacgtcaaaaagggtggagccaagaaaagacccgcccccagtgacgcagatataagtgagcccaaacgggtgcgcgagtcagttgcgcagccatcgacgtcagacgcggaagcttcgatcaactacgcagacaggtaccaaaacaaatgttctcgtcacgtgggcatgaatctgatgctgtttccctgcagacaatgcgagagaatgaatcagaattcaaatatctgcttcactcacggacagaaagactgtttagagtgctttcccgtgtcagaatctcaacccgtttctgtcgtcaaaaaggcgtatcagaaactgtgctacattcatcatatcatgggaaaggtgccagacgcttgcactgcctgcgatctggtcaatgtggatttggatgactgcatctttgaacaataaatgatttaaatcaggtatggctgccgatggttatcttccagattggctcgaggacaacctctctgagggcattcgcgagtggtgggcgctgaaacctggagccccgaagcccaaagccaaccagcaaaagcaggacgacggccggggtctggtgcttcctggctacaagtacctcggacccttcaacggactcgacaagggggagcccgtcaacgcggcggacgcagcggccctcgagcacgacaaggcctacgaccagcagctgcaggcgggtgacaatccgtacctgcggtataaccacgccgacgccgagtttcaggagcgtctgcaagaagatacgtcttttgggggcaacctcgggcgagcagtcttccaggccaagaagcgggttctcgaacctctcggtctggttgaggaaggcgctaagacggctcctggaaagaagagaccggtagagccatcaccccagcgttctccagactcctctacgggcatcggcaagaaaggccaacagcccgccagaaaaagactcaattttggtcagactggcgactcagagtcagttccagaccctcaacctctcggagaacctccagcagcgccctctggtgtgggacctaatacaatggctgcaggcggtggcgcaccaatggcagacaataacgaaggcgccgacggagtgggtagttcctcgggaaattggcattgcgattccacatggctgggcgacagagtcatcaccaccagcacccgaacctgggccctgcccacctacaacaaccacctctacaagcaaatctccaacgggacatcgggaggagccaccaacgacaacacctacttcggctacagcaccccctgggggtattttgactttaacagattccactgccacttttcaccacgtgactggcagcgactcatcaacaacaactggggattccggcccaagagactcagcttcaagctcttcaacatccaggtcaaggaggtcacgcagaatgaaggcaccaagaccatcgccaataacctcaccagcaccatccaggtgtttacggactcggagtaccagctgccgtacgttctcggctctgcccaccagggctgcctgcctccgttcccggcggacgtgttcatgattccccagtacggctacctaacactcaacaacggtagtcaggccgtgggacgctcctccttctactgcctggaatactttccttcgcagatgctgagaaccggcaacaacttccagtttacttacaccttcgaggacgtgcctttccacagcagctacgcccacagccagagcttggaccggctgatgaatcctctgattgaccagtacctgtactacttgtctcggactcaaacaacaggaggcacggcaaatacgcagactctgggcttcagccaaggtgggcctaatacaatggccaatcaggcaaagaactggctgccaggaccctgttaccgccaacaacgcgtctcaacgacaaccgggcaaaacaacaatagcaactttgcctggactgctgggaccaaataccatctgaatggaagaaattcattggctaatcctggcatcgctatggcaacacacaaagacgacgaggagcgtttttttcccagtaacgggatcctgatttttggcaaacaaaatgctgccagagacaatgcggattacagcgatgtcatgctcaccagcgaggaagaaatcaaaaccactaaccctgtggctacagaggaatacggtatcgtggcagataacttgcagcagcaaaacacggctcctcaaattggaactgtcaacagccagggggccttacccggtatggtctggcagaaccgggacgtgtacctgcagggtcccatctgggccaagattcctcacacggacggcaacttccacccgtctccgctgatgggcggctttggcctgaaacatcctccgcctcagatcctgatcaagaacacgcctgtacctgcggatcctccgaccaccttcaaccagtcaaagctgaactctttcatcacgcaatacagcaccggacaggtcagcgtggaaattgaatgggagctgcagaaggaaaacagcaagcgctggaaccccgagatccagtacacctccaactactacaaatctacaagtgtggactttgctgttaatacagaaggcgtgtactctgaaccccgccccattggcacccgttacctcacccgtaatctgtaattgcctgttaatcaataaaccgtttaattcgtttcagttgaactttggtctctgcgtatttctttcttatctagtttccatggctacgtagataagtagcatggcgggttaatcattaactacagcccgggcgtttaaacagcgggcggaggggtggagtcgtgacgtgaattacgtcatagggttagggaggtcctgtattagaggtcacgtgagtgttttgcgacattttgcgacaccatgtggtctcgctgggggggggggcccgagtgagcacgcagggtctccattttgaagcgggaggtttgaacgagcgctggcgcgctcactggccgtcgttttacaacgtcgtgactgggaaaaccctggcgttacccaacttaatcgccttgcagcacatccccctttcgccagctggcgtaatagcgaagaggcccgcaccgatcgcccttcccaacagttgcgcagcctgaatggcgaatggaaattgtaagcgttaatattttgttaaaattcgcgttaaatttttgttaaatcagctcatttttttaaccaataggccgaaatcggcaaaatcccttataaatcaaaagaatagaccgagatagggttgagtgttgttccagtttggaacaagagtccactattaagaacgtggactccaacgtcaaagggcgaaaaaccgtctatcagggcgatggcccactacgtgaaccatcaccctaatcaagttttttggggtcgaggtgccgtaaagcactaaatcggaaccctaaagggagcccccgatttagagcttgacggggaaagccggcgaacgtggcgagaaaggaagggaagaaagcgaaaggagcgggcgctagggcgctggcaagtgtagcggtcacgctgcgcgtaaccaccacacccgccgcgcttaatgcgccgctacagggcgcgtcaggtggcacttttcggggaaatgtgcgcggaacccctatttgtttatttttctaaatacattcaaatatgtatccgctcatgagacaataaccctgataaatgcttcaataatattgaaaaaggaagagtatgagtattcaacatttccgtgtcgcccttattcccttttttgcggcattttgccttcctgtttttgctcacccagaaacgctggtgaaagtaaaagatgctgaagatcagttgggtgcacgagtgggttacatcgaactggatctcaacagcggtaagatccttgagagttttcgccccgaagaacgttttccaatgatgagcacttttaaagttctgctatgtggcgcggtattatcccgtattgacgccgggcaagagcaactcggtcgccgcatacactattctcagaatgacttggttgagtactcaccagtcacagaaaagcatcttacggatggcatgacagtaagagaattatgcagtgctgccataaccatgagtgataacactgcggccaacttacttctgacaacgatcggaggaccgaaggagctaaccgcttttttgcacaacatgggggatcatgtaactcgccttgatcgttgggaaccggagctgaatgaagccataccaaacgacgagcgtgacaccacgatgcctgtagcaatggcaacaacgttgcgcaaactattaactggcgaactacttactctagcttcccggcaacaattaatagactggatggaggcggataaagttgcaggaccacttctgcgctcggcccttccggctggctggtttattgctgataaatctggagccggtgagcgtgggtctcgcggtatcattgcagcactggggccagatggtaagccctcccgtatcgtagttatctacacgacggggagtcaggcaactatggatgaacgaaatagacagatcgctgagataggtgcctcactgattaagcattggtaactgtcagaccaagtttactcatatatactttagattgatttaaaacttcatttttaatttaaaaggatctaggtgaagatcctttttgataatctcatgaccaaaatcccttaacgtgagttttcgttccactgagcgtcagaccccgtagaaaagatcaaaggatcttcttgagatcctttttttctgcgcgtaatctgctgcttgcaaacaaaaaaaccaccgctaccagcggtggtttgtttgccggatcaagagctaccaactctttttccgaaggtaactggcttcagcagagcgcagataccaaatactgttcttctagtgtagccgtagttaggccaccacttcaagaactctgtagcaccgcctacatacctcgctctgctaatcctgttaccagtggctgctgccagtggcgataagtcgtgtcttaccgggttggactcaagacgatagttaccggataaggcgcagcggtcgggctgaacggggggttcgtgcacacagcccagcttggagcgaacgacctacaccgaactgagatacctacagcgtgagctatgagaaagcgccacgcttcccgaagggagaaaggcggacaggtatccggtaagcggcagggtcggaacaggagagcgcacgagggagcttccagggggaaacgcctggtatctttatagtcctgtcgggtttcgccacctctgacttgagcgtcgatttttgtgatgctcgtcaggggggcggagcctatggaaaaacgccagcaacgcggcctttttacggttcctggccttttgctggccttttgctcacatgttctttcctgcgttatcccctgattctgtggataaccgtattaccgcctttgagtgagctgataccgctcgccgcagccgaacgaccgagcgcagcgagtcagtgagcgaggaagcggaagagcgcccaatacgcaaaccgcctctccccgcgcgttggccgattcattaatgcagctggcacgacaggtttcccgactggaaagcgggcagtgagcgcaacgcaattaatgtgagttagctcactcattaggcaccccaggctttacactttatgcttccggctcgtatgttgtgtggaattgtgagcggataacaatttcacacaggaaacagctatgaccatgattacgccaa

SEQ ID NO: 24 - DNA, 7366 bp, Artificial Sequence
  paav RC2/8 myc plasmid
gcgcgccgatatcgttaacgccccgcgccggccgctctagaactagtggatcccccggaagatcagaagttcctattccgaagttcctattctctagaaagtataggaacttctgatctgcgcagccgccatgccggggttttacgagattgtgattaaggtccccagcgaccttgacgagcatctgcccggcatttctgacagctttgtgaactgggtggccgagaaggaatgggagttgccgccagattctgacatggatctgaatctgattgagcaggcacccctgaccgtggccgagaagctgcagcgcgactttctgacggaatggcgccgtgtgagtaaggccccggaggcccttttctttgtgcaatttgagaagggagagagctacttccacatgcacgtgctcgtggaaaccaccggggtgaaatccatggttttgggacgtttcctgagtcagattcgcgaaaaactgattcagagaatttaccgcgggatcgagccgactttgccaaactggttcgcggtcacaaagaccagaaatggcgccggaggcgggaacaaggtggtggatgagtgctacatccccaattacttgctccccaaaacccagcctgagctccagtgggcgtggactaatatggaacagtatttaagcgcctgtttgaatctcacggagcgtaaacggttggtggcgcagcatctgacgcacgtgtcgcagacgcaggagcagaacaaagagaatcagaatcccaattctgatgcgccggtgatcagatcaaaaacttcagccaggtacatggagctggtcgggtggctcgtggacaaggggattacctcggagaagcagtggatccaggaggaccaggcctcatacatctccttcaatgcggcctccaactcgcggtcccaaatcaaggctgccttggacaatgcgggaaagattatgagcctgactaaaaccgcccccgactacctggtgggccagcagcccgtggaggacatttccagcaatcggatttataaaattttggaactaaacgggtacgatccccaatatgcggcttccgtctttctgggatgggccacgaaaaagttcggcaagaggaacaccatctggctgtttgggcctgcaactaccgggaagaccaacatcgcggaggccatagcccacactgtgcccttctacgggtgcgtaaactggaccaatgagaactttcccttcaacgactgtgtcgacaagatggtgatctggtgggaggaggggaagatgaccgccaaggtcgtggagtcggccaaagccattctcggaggaagcaaggtgcgcgtggaccagaaatgcaagtcctcggcccagatagacccgactcccgtgatcgtcacctccaacaccaacatgtgcgccgtgattgacgggaactcaacgaccttcgaacaccagcagccgttgcaagaccggatgttcaaatttgaactcacccgccgtctggatcatgactttgggaaggtcaccaagcaggaagtcaaagactttttccggtgggcaaaggatcacgtggttgaggtggagcatgaattctacgtcaaaaagggtggagccaagaaaagacccgcccccagtgacgcagatataagtgagcccaaacgggtgcgcgagtcagttgcgcagccatcgacgtcagacgcggaagcttcgatcaactacgcagacaggtaccaaaacaaatgttctcgtcacgtgggcatgaatctgatgctgtttccctgcagacaatgcgagagaatgaatcagaattcaaatatctgcttcactcacggacagaaagactgtttagagtgctttcccgtgtcagaatctcaacccgtttctgtcgtcaaaaaggcgtatcagaaactgtgctacattcatcatatcatgggaaaggtgccagacgcttgcactgcctgcgatctggtcaatgtggatttggatgactgcatctttgaacaataaatgatttaaatcaggtatggctgccgatggttatcttccagattggctcgaggacaacctctctgagggcattcgcgagtggtgggcgctgaaacctggagccccgaagcccaaagccaaccagcaaaagcaggacgacggccggggtctggtgcttcctggctacaagtacctcggacccttcaacggactcgacaagggggagcccgtcaacgcggcggacgcagcggccctcgagcacgacaaggcctacgaccagcagctgcaggcgggtgacaatccgtacctgcggtataaccacgccgacgccgagtttcaggagcgtctgcaagaagatacgtcttttgggggcaacctcgggcgagcagtcttccaggccaagaagcgggttctcgaacctctcggtctggttgaggaaggcgctaagacggctcctggaaagaagagaccggtagagccatcaccccagcgttctccagactcctctacgggcatcggcaagaaaggccaacagcccgccagaaaaagactcaattttggtcagactggcgactcagagtcagttccagaccctcaacctctcggagaacctccagcagcgccctctggtgtgggacctaatacaatggctgcaggcggtggcgcaccaatggcagacaataacgaaggcgccgacggagtgggtagttcctcgggaaattggcattgcgattccacatggctgggcgacagagtcatcaccaccagcacccgaacctgggccctgcccacctacaacaaccacctctacaagcaaatctccaacgggacatcgggaggagccaccaacgacaacacctacttcggctacagcaccccctgggggtattttgactttaacagattccactgccacttttcaccacgtgactggcagcgactcatcaacaacaactggggattccggcccaagagactcagcttcaagctcttcaacatccaggtcaaggaggtcacgcagaatgaaggcaccaagaccatcgccaataacctcaccagcaccatccaggtgtttacggactcggagtaccagctgccgtacgttctcggctctgcccaccagggctgcctgcctccgttcccggcggacgtgttcatgattccccagtacggctacctaacactcaacaacggtagtcaggccgtgggacgctcctccttctactgcctggaatactttccttcgcagatgctgagaaccggcaacaacttccagtttacttacaccttcgaggacgtgcctttccacagcagctacgcccacagccagagcttggaccggctgatgaatcctctgattgaccagtacctgtactacttgtctcggactcaaacaacaggaggcacggcaaatacgcagactctgggcttcagccaaggtgggcctaatacaatggccaatcaggcaaagaactggctgccaggaccctgttaccgccaacaacgcgtctcaacgacaaccgggcaaaacaacaatagcaactttgcctggactgctgggaccaaataccatctgaatggaagaaattcattggctaatcctggcatcgctatggcaacacacaaagacgacgaggagcgtttttttcccagtaacgggatcctgatttttggcaaacaaaatgctgccagagacaatgcggattacagcgatgtcatgctcaccagcgaggaagaaatcaaaaccactaaccctgtggctacagaggaatacggtatcgtggcagataacttgcagcagcaaaacgaacaaaaactcatctcagaagaggatctgacggctcctcaaattggaactgtcaacagccagggggccttacccggtatggtctggcagaaccgggacgtgtacctgcagggtcccatctgggccaagattcctcacacggacggcaacttccacccgtctccgctgatgggcggctttggcctgaaacatcctccgcctcagatcctgatcaagaacacgcctgtacctgcggatcctccgaccaccttcaaccagtcaaagctgaactctttcatcacgcaatacagcaccggacaggtcagcgtggaaattgaatgggagctgcagaaggaaaacagcaagcgctggaaccccgagatccagtacacctccaactactacaaatctacaagtgtggactttgctgttaatacagaaggcgtgtactctgaaccccgccccattggcacccgttacctcacccgtaatctgtaattgcctgttaatcaataaaccgtttaattcgtttcagttgaactttggtctctgcgtatttctttcttatctagtttccatggctacgtagataagtagcatggcgggttaatcattaactacagcccgggcgtttaaacagcgggcggaggggtggagtcgtgacgtgaattacgtcatagggttagggaggtcctgtattagaggtcacgtgagtgttttgcgacattttgcgacaccatgtggtctcgctgggggggggggcccgagtgagcacgcagggtctccattttgaagcgggaggtttgaacgagcgctggcgcgctcactggccgtcgttttacaacgtcgtgactgggaaaaccctggcgttacccaacttaatcgccttgcagcacatccccctttcgccagctggcgtaatagcgaagaggcccgcaccgatcgcccttcccaacagttgcgcagcctgaatggcgaatggaaattgtaagcgttaatattttgttaaaattcgcgttaaatttttgttaaatcagctcatttttttaaccaataggccgaaatcggcaaaatcccttataaatcaaaagaatagaccgagatagggttgagtgttgttccagtttggaacaagagtccactattaagaacgtggactccaacgtcaaagggcgaaaaaccgtctatcagggcgatggcccactacgtgaaccatcaccctaatcaagttttttggggtcgaggtgccgtaaagcactaaatcggaaccctaaagggagcccccgatttagagcttgacggggaaagccggcgaacgtggcgagaaaggaagggaagaaagcgaaaggagcgggcgctagggcgctggcaagtgtagcggtcacgctgcgcgtaaccaccacacccgccgcgcttaatgcgccgctacagggcgcgtcaggtggcacttttcggggaaatgtgcgcggaacccctatttgtttatttttctaaatacattcaaatatgtatccgctcatgagacaataaccctgataaatgcttcaataatattgaaaaaggaagagtatgagtattcaacatttccgtgtcgcccttattcccttttttgcggcattttgccttcctgtttttgctcacccagaaacgctggtgaaagtaaaagatgctgaagatcagttgggtgcacgagtgggttacatcgaactggatctcaacagcggtaagatccttgagagttttcgccccgaagaacgttttccaatgatgagcacttttaaagttctgctatgtggcgcggtattatcccgtattgacgccgggcaagagcaactcggtcgccgcatacactattctcagaatgacttggttgagtactcaccagtcacagaaaagcatcttacggatggcatgacagtaagagaattatgcagtgctgccataaccatgagtgataacactgcggccaacttacttctgacaacgatcggaggaccgaaggagctaaccgcttttttgcacaacatgggggatcatgtaactcgccttgatcgttgggaaccggagctgaatgaagccataccaaacgacgagcgtgacaccacgatgcctgtagcaatggcaacaacgttgcgcaaactattaactggcgaactacttactctagcttcccggcaacaattaatagactggatggaggcggataaagttgcaggaccacttctgcgctcggcccttccggctggctggtttattgctgataaatctggagccggtgagcgtgggtctcgcggtatcattgcagcactggggccagatggtaagccctcccgtatcgtagttatctacacgacggggagtcaggcaactatggatgaacgaaatagacagatcgctgagataggtgcctcactgattaagcattggtaactgtcagaccaagtttactcatatatactttagattgatttaaaacttcatttttaatttaaaaggatctaggtgaagatcctttttgataatctcatgaccaaaatcccttaacgtgagttttcgttccactgagcgtcagaccccgtagaaaagatcaaaggatcttcttgagatcctttttttctgcgcgtaatctgctgcttgcaaacaaaaaaaccaccgctaccagcggtggtttgtttgccggatcaagagctaccaactctttttccgaaggtaactggcttcagcagagcgcagataccaaatactgttcttctagtgtagccgtagttaggccaccacttcaagaactctgtagcaccgcctacatacctcgctctgctaatcctgttaccagtggctgctgccagtggcgataagtcgtgtcttaccgggttggactcaagacgatagttaccggataaggcgcagcggtcgggctgaacggggggttcgtgcacacagcccagcttggagcgaacgacctacaccgaactgagatacctacagcgtgagctatgagaaagcgccacgcttcccgaagggagaaaggcggacaggtatccggtaagcggcagggtcggaacaggagagcgcacgagggagcttccagggggaaacgcctggtatctttatagtcctgtcgggtttcgccacctctgacttgagcgtcgatttttgtgatgctcgtcaggggggcggagcctatggaaaaacgccagcaacgcggcctttttacggttcctggccttttgctggccttttgctcacatgttctttcctgcgttatcccctgattctgtggataaccgtattaccgcctttgagtgagctgataccgctcgccgcagccgaacgaccgagcgcagcgagtcagtgagcgaggaagcggaagagcgcccaatacgcaaaccgcctctccccgcgcgttggccgattcattaatgcagctggcacgacaggtttcccgactggaaagcgggcagtgagcgcaacgcaattaatgtgagttagctcactcattaggcaccccaggctttacactttatgcttccggctcgtatgttgtgtggaattgtgagcggataacaatttcacacaggaaacagctatgaccatgattacgccaa

SEQ ID NO: 25 - protein, 748 aa, Artificial Sequence
  pAAV8N590myc
MAADGYLPDWLEDNLSEGIREWWALKPGAPKPKANQQKQDDGRGLVLPGYKYLGPFNGLDKGEPVNAADAAALEHDKAYDQQLQAGDNPYLRYNHADAEFQERLQEDTSFGGNLGRAVFQAKKRVLEPLGLVEEGAKTAPGKKRPVEPSPQRSPDSSTGIGKKGQQPARKRLNFGQTGDSESVPDPQPLGEPPAAPSGVGPNTMAAGGGAPMADNNEGADGVGSSSGNWHCDSTWLGDRVITTSTRTWALPTYNNHLYKQISNGTSGGATNDNTYFGYSTPWGYFDFNRFHCHFSPRDWQRLINNNWGFRPKRLSFKLFNIQVKEVTQNEGTKTIANNLTSTIQVFTDSEYQLPYVLGSAHQGCLPPFPADVFMIPQYGYLTLNNGSQAVGRSSFYCLEYFPSQMLRTGNNFQFTYTFEDVPFHSSYAHSQSLDRLMNPLIDQYLYYLSRTQTTGGTANTQTLGFSQGGPNTMANQAKNWLPGPCYRQQRVSTTTGQNNNSNFAWTAGTKYHLNGRNSLANPGIAMATHKDDEERFFPSNGILIFGKQNAARDNADYSDVMLTSEEEIKTTNPVATEEYGIVADNLQQQNEQKLISEEDLTAPQIGTVNSQGALPGMVWQNRDVYLQGPIWAKIPHTDGNFHPSPLMGGFGLKHPPPQILIKNTPVPADPPTTFNQSKLNSFITQYSTGQVSVEIEWELQKENSKRWNPEIQYTSNYYKSTSVDFAVNTEGVYSEPRPIGTRYLTRNL

SEQ ID NO: 26 - protein, 746 aa, Artificial Sequence
  pAAV9A589myc
MAADGYLPDWLEDNLSEGIREWWALKPGAPQPKANQQHQDNARGLVLPGYKYLGPGNGLDKGEPVNAADAAALEHDKAYDQQLKAGDNPYLKYNHADAEFQERLKEDTSFGGNLGRAVFQAKKRLLEPLGLVEEAAKTAPGKKRPVEQSPQEPDSSAGIGKSGAQPAKKRLNFGQTGDTESVPDPQPIGEPPAAPSGVGSLTMASGGGAPVADNNEGADGVGSSSGNWHCDSQWLGDRVITTSTRTWALPTYNNHLYKQISNSTSGGSSNDNAYFGYSTPWGYFDFNRFHCHFSPRDWQRLINNNWGFRPKRLNFKLFNIQVKEVTDNNGVKTIANNLTSTVQVFTDSDYQLPYVLGSAHEGCLPPFPADVFMIPQYGYLTLNDGSQAVGRSSFYCLEYFPSQMLRTGNNFQFSYEFENVPFHSSYAHSQSLDRLMNPLIDQYLYYLSKTINGSGQNQQTLKFSVAGPSNMAVQGRNYIPGPSYRQQRVSTTVTQNNNSEFAWPGASSWALNGRNSLMNPGPAMASHKEGEDRFFPLSGSLIFGKQGTGRDNVDADKVMITNEEEIKTTNPVATESYGQVATNHQSAQAEQKLISEEDLQAQTGWVQNQGILPGMVWQDRDVYLQGPIWAKIPHTDGNFHPSPLMGGFGMKHPPPQILIKNTPVPADPPTAFNKDKLNSFITQYSTGQVSVEIEWELQKENSKRWNPEIQYTSNYYKSNNVEFAVNTEGVYSEPRPIGTRYLTRNL

SEQ ID NO: 27 - protein, 746 aa, Artificial Sequence
  pAAV9G453myc
MAADGYLPDWLEDNLSEGIREWWALKPGAPQPKANQQHQDNARGLVLPGYKYLGPGNGLDKGEPVNAADAAALEHDKAYDQQLKAGDNPYLKYNHADAEFQERLKEDTSFGGNLGRAVFQAKKRLLEPLGLVEEAAKTAPGKKRPVEQSPQEPDSSAGIGKSGAQPAKKRLNFGQTGDTESVPDPQPIGEPPAAPSGVGSLTMASGGGAPVADNNEGADGVGSSSGNWHCDSQWLGDRVITTSTRTWALPTYNNHLYKQISNSTSGGSSNDNAYFGYSTPWGYFDFNRFHCHFSPRDWQRLINNNWGFRPKRLNFKLFNIQVKEVTDNNGVKTIANNLTSTVQVFTDSDYQLPYVLGSAHEGCLPPFPADVFMIPQYGYLTLNDGSQAVGRSSFYCLEYFPSQMLRTGNNFQFSYEFENVPFHSSYAHSQSLDRLMNPLIDQYLYYLSKTINGEQKLISEEDLSGQNQQTLKFSVAGPSNMAVQGRNYIPGPSYRQQRVSTTVTQNNNSEFAWPGASSWALNGRNSLMNPGPAMASHKEGEDRFFPLSGSLIFGKQGTGRDNVDADKVMITNEEEIKTTNPVATESYGQVATNHQSAQAQAQTGWVQNQGILPGMVWQDRDVYLQGPIWAKIPHTDGNFHPSPLMGGFGMKHPPPQILIKNTPVPADPPTAFNKDKLNSFITQYSTGQVSVEIEWELQKENSKRWNPEIQYTSNYYKSNNVEFAVNTEGVYSEPRPIGTRYLTRNL

SEQ ID NO: 28 - DNA, 814 bp, Artificial Sequence
  cmyc-scfv-gblock
tctccctgtctctgggtaaaggcggaggtggatccggagggggcggatctgacatccagatgacccagtctccatcctccctgtctgcatctgtaggagacagagtcaccatcacttgccgggcaagtcagagcattagcagctatttaaattggtatcaacagaaaccagggaaagcccctaagctcctgatctatgctgtttccattttgcaaagtggggtcccatcaaggttcagtggcagtggatctgggacagatttcactctcaccatcaactctctgcaacctgaagattttgcaacttactcctgtcaacagacttacagtacccctccgatcaccttcggccaagggacacgactggagattaaaggagggggcggctcaggaggagggggtagtgggggaggcggctccgaggtgcagctggtggagtctgggggaggcttggtacagcctggagggtccctgagactctcctgtgtcacctctggatttcgttttagtagttatgaaatgaactgggtccgccaggctccagggaaggggctggaatggatttcatacattaacagaagtggttataccatatactacgcagcctctctgaagggccgattcaccatctccagagacaacgccaagaactcactgtatcttcaaatgaacagcctgagagacgaggacacggctatctattactgtgcgagagggagtatcgcccctcggggggagattcgacacatctttgactactggggccagggaaccctggtcaccgtctcctcatgatgagcggccgctaatcagcc

SEQ ID NO: 29 - protein, 120 aa, Artificial Sequence
  myc HCVR AA
EVQLVESGGGLVQPGGSLRLSCVTSGFRFSSYEMNWVRQAPGKGLEWISYINRSGYTIYYAASLKGRFTISRDNAKNSLYLQMNSLRDEDTAIYYCARGSIAPRGEIRHIFDYWGQGTLV

SEQ ID NO: 30 - protein, 108 aa, Artificial Sequence
  myc LCVR AA
DIQMTQSPSSLSASVGDRVTITCRASQSISSYLNWYQQKPGKAPKLLIYAASSLQSGVPSRFSGSGSGTDFTLTISSLQPEDFATYYCQQSYSTPPITFGQGTRLEIK

SEQ ID NO: 31 - protein, 8 aa, Artificial Sequence
  myc HCDR1
GFRFSSYE

SEQ ID NO: 32 - protein, 8 aa, Artificial Sequence
  myc HCDR2 AA
INRSGYTI

SEQ ID NO: 33 - protein, 2 aa, Artificial Sequence
  myc HCDR3
AR

SEQ ID NO: 34 - protein, 6 aa, Artificial Sequence
  myc LCDR1 AA
QSISSY

SEQ ID NO: 35 - protein, 3 aa, Artificial Sequence
  myc LCDR2
AAS

SEQ ID NO: 36 - protein, 7 aa, Artificial Sequence
  myc LCDR3 AA
QQSYSTP

SEQ ID NO: 37 - protein, 247 aa, Artificial Sequence
  anti-myc scFv
DIQMTQSPSSLSASVGDRVTITCRASQSISSYLNWYQQKPGKAPKLLIYAVSILQSGVPSRFSGSGSGTDFTLTINSLQPEDFATYSCQQTYSTPPITFGQGTRLEIKGGGGSGGGGSGGGGSEVQLVESGGGLVQPGGSLRLSCVTSGFRFSSYEMNWVRQAPGKGLEWISYINRSGYTIYYAASLKGRFTISRDNAKNSLYLQMNSLRDEDTAIYYCARGSIAPRGEIRHIFDYWGQGTLVTVSS

SEQ ID NO: 38 - DNA, 774 bp, Artificial Sequence
  anti-myc scFv NA
ggcggaggtggatccggagggggcggatctgacatccagatgacccagtctccatcctccctgtctgcatctgtaggagacagagtcaccatcacttgccgggcaagtcagagcattagcagctatttaaattggtatcaacagaaaccagggaaagcccctaagctcctgatctatgctgtttccattttgcaaagtggggtcccatcaaggttcagtggcagtggatctgggacagatttcactctcaccatcaactctctgcaacctgaagattttgcaacttactcctgtcaacagacttacagtacccctccgatcaccttcggccaagggacacgactggagattaaaggagggggcggctcaggaggagggggtagtgggggaggcggctccgaggtgcagctggtggagtctgggggaggcttggtacagcctggagggtccctgagactctcctgtgtcacctctggatttcgttttagtagttatgaaatgaactgggtccgccaggctccagggaaggggctggaatggatttcatacattaacagaagtggttataccatatactacgcagcctctctgaagggccgattcaccatctccagagacaacgccaagaactcactgtatcttcaaatgaacagcctgagagacgaggacacggctatctattactgtgcgagagggagtatcgcccctcggggggagattcgacacatctttgactactggggccagggaaccctggtcaccgtctcctcatga

SEQ ID NO: 39 - DNA, 372 bp, Artificial Sequence
  myc HCVR NA
gaggtgcagctggtggagtctgggggaggcttggtacagcctggagggtccctgagactctcctgtgtcacctctggatttcgttttagtagttatgaaatgaactgggtccgccaggctccagggaaggggctggaatggatttcatacattaacagaagtggttataccatatactacgcagcctctctgaagggccgattcaccatctccagagacaacgccaagaactcactgtatcttcaaatgaacagcctgagagacgaggacacggctatctattactgtgcgagagggagtatcgcccctcggggggagattcgacacatctttgactactggggccagggaaccctggtcaccgtctcctca

SEQ ID NO: 40 - DNA, 324 bp, Artificial Sequence
  myc LCVR NA
gacatccagatgacccagtctccatcctccctgtctgcatctgtaggagacagagtcaccatcacttgccgggcaagtcagagcattagcagctatttaaattggtatcagcagaaaccagggaaagcccctaagctcctgatctatgctgcatccagtttgcaaagtggggtcccgtcaaggttcagtggcagtggatctgggacagatttcactctcaccatcagcagtctgcaacctgaagattttgcaacttactactgtcaacagagttacagtacccctccgatcaccttcggccaagggacacgactggagattaaa